European Patent Specification EP 4 204 551 B1, published September 17, 2025. Title: VARIANTS OF A FAMILY 44 XYLOGLUCANASE. Applicant: NOVOZYMES A/S. The sequence listing filed with the application follows.

SEQUENCE LISTING (4 sequences)

SEQ ID NO: 1 - protein, 524 aa, Paenibacillus polymyxa
VVHGQTAKTITIKVDTFKDRKPISPYIYGTNQDLAGDENMAARRLGGNRMTGYNWENNMSNAGSDWQQSSDNYLCSNGGLTQAECEKPGAVTTSFHDQSLKLGTYSLVTLPMAGYVAKDGNGSVQESEKAPSARWNQVVNAKNAPFQLQPDLNDNRVYVDEFVHFLVNKYGTASTKAGVKGYALDNEPALWSHTHPRIHGEKVGAKELVDRSVSLSKAVKAIDAGAEVFGPVLYGFGAYKDLQTAPDWDSVKGNYSWFVDYYLDQMRLSSQVEGKRLLDVFDVHWYPEAMGGGIRITNEVGNDETKKARMQAPRTLWDPTYKEDSWIAQWNSEFLPILPRLKQSVDKYYPGTKLAMTEYSYGGENDISGGIAMTDVLGILGKNDVYMANYWKLKDGVNNYVSAAYKLYRNYDGKNSTFGDTSVSAQTSDIVNSSVHASVTNASDKELHLVVMNKSMDSAFDAQFDLSGAKTYISGKVWGFDKNSSQIKEAAPITQISGNRFTYTVPPLTAYHIVLTTGNDTSPV

SEQ ID NO: 2 - protein, 524 aa, Artificial
  Synthetic Construct
VVHGQTAKTITIKVDTFKDRKPISPYIYGTNQDLAGDENMAARRLGGNRMTGYNWENNMSNAGSDWQHSSDNYLCSNGGLTQAECEKPGAVVTSFHDQSLKLGTYSLVTLPMAGYVAADGNGSVQESEAAPSARWNQVVNAKNAPFQLQPDLNDNYVYVDEFVHFLVNKYGTASTKAGVKGYALDNEPALWSHTHPRIHPEKVGAKELVDRSVSLSKAVKAIDAGAEVFGPVLYGFGAYKDLQTAPDWDSVKGNYSWFVDYYLDQMRLSSQVEGKRLLDVFDVHWYPEAMGGGIRITNEVGNDETKKARMQAPRTLWDPTYKEDSWIAQWFSEFLPILPRLKQSVDKYYPGTKLAMTEYSYGGENDISGGIAMTDVLGILGKNDVYMANYWKLKDGVNNYVSAAYKLYRNYDGKNSTFGDTSVSAQTSDIVNSSVHASVTNASDKELHLVVMNKSMDSAFDAQFDLSGAKTYISGKVWGFDKNSSQIKEAAPITQISGNRFTYTVPPLTAYHIVLTTGNDTSPV

SEQ ID NO: 3 - protein, 524 aa, Artificial Sequence
  Synthetic Construct
VVHGQTAKTITIKVDTFKDRKPISPYIYGTNQDLAGDENMAARRLGGNRMTGYNWENNMSNAGSDWQHSSDNYLCSNGGLTQAECEKPGAVVTSFHDQSLKLGTYSLVTLPMAGYVAADGNGSVQESETAPSARWNQVVNAKNAPFQLQPDLNDNYVYVDEFVHFLVNKYGTASTKAGVKGYALDNEPALWSHTHPRIHPEKVGAKELVDRSVSLSKAVKAIDAGAEVFGPVLYGFGAYKDLQTAPDWDSVKGNYSWFVDYYLDQMRLSSQVEGKRLLDVFDVHWYPEAMGGGIRITNEVGNDETKKARMQAPRTLWDPTYKEDSWIAQWFSEFLPILPRLKQSVDKYYPGTKLAMTEYSYGGENDISGGIAMTDVLGILGKNDVYMANYWKLKDGVNNYVSAAYKLYRNYDGKNSTFGDTSVSAQTSDIVNSSVHASVTNASDKELHLVVMNKSMDSAFDAQFDLSGAKTYISGKVWGFDKNSSQIKEAAPITQISGNRFTYTVPPLTAYHIVLTTGNDTSPV

SEQ ID NO: 4 - protein, 269 aa, Bacillus lentus
AQSVPWGISRVQAPAAHNRGLTGSGVKVAVLDTGISTHPDLNIRGGASFVPGEPSTQDGNGHGTHVAGTIAALNNSIGVLGVAPSAELYAVKVLGASGSGSVSSIAQGLEWAGNNGMHVANLSLGSPSPSATLEQAVNSATSRGVLVVAASGNSGAGSISYPARYANAMAVGATDQNNNRASFSQYGAGLDIVAPGVNVQSTYPGSTYASLNGTSMATPHVAGAAALVKQKNPSWSNVQIRNHLKNTATSLGSTNLYGSGLVNAEAATR